European Patent Application EP 4 332 120 A1, published March 6, 2024. Title: BISPECIFIC ANTIBODY-DRUG CONJUGATE. Applicant: XUANZHU BIOPHARMACEUTICAL CO., LTD. BEIJING XUANZHU COMBIO CO., LTD. Application EP22794892.4. The sequence listing filed with the application follows.

SEQUENCE LISTING (16 sequences)

SEQ ID NO: 1 - protein, 107 aa, Artificial Sequence [sequence omitted]

SEQ ID NO: 2 - protein, 214 aa, Artificial Sequence
  Synthetic polypeptide
DIQMTQSPSSLSASVGDRVTITCKASQDVSIGVAWYQQKPGKAPKLLIYSASYRYTGVPSRFSGSGSGTDFTLTISSLQPEDFATYYCQQYYIYPYTFGQGTKVEIKRTVAAPSVFIFPPSDEQLKSGTASVVCLLNNFYPREAKVQWKVDNALQSGNSQESVTEQDSKDSTYSLSSTLTLSKADYEKHKVYACEVTHQGLSSPVTKSFNRGEC

SEQ ID NO: 3 - protein, 119 aa, Artificial Sequence [sequence omitted]

SEQ ID NO: 4 - protein, 448 aa, Artificial Sequence
  Synthetic polypeptide
EVQLVESGGGLVQPGGSLRLSCAASGFTFTDYTMDWVRQAPGKGLEWVADVNPNSGGSIYNQRFKGRFTLSVDRSKNTLYLQMNSLRAEDTAVYYCARNLGPSFYFDYWGQGTLVTVSSASTKGPSVFPLAPSSKSTSGGTAALGCLVKDYFPEPVTVSWNSGALTSGVHTFPAVLQSSGLYSLSSVVTVPSSSLGTQTYICNVNHKPSNTKVDKKVEPKSCDKTHTCPPCPAPELLGGPSVFLFPPKPKDTLMISRTPEVTCVVVDVSHEDPEVKFNWYVDGVEVHNAKTKPREEQYNSTYRVVSVLTVLHQDWLNGKEYKCKVSNKALPAPIEKTISKAKGQPREPQVYTLPPSREEMTKNQVSLTCLVKGFYPSDIAVEWESNGQPENNYKTTPPVLDSDGSFFLYSKLTVDKSRWQQGNVFSCSVMHEALHNHYTQKSLSLSPG

SEQ ID NO: 5 - protein, 107 aa, Artificial Sequence [sequence omitted]

SEQ ID NO: 6 - protein, 214 aa, Artificial Sequence
  Synthetic polypeptide
DIQMTQSPSSLSASVGDRVTITCRASQDVNTAVAWYQQKPGKAPKLLIYSASFLYSGVPSRFSGSRSGTDFTLTISSLQPEDFATYYCQQHYTTPPTFGQGTKVEIKRTVAAPSVFIFPPSDEQLKSGTASVVCLLNNFYPREAKVQWKVDNALQSGNSQESVTEQDSKDSTYSLSSTLTLSKADYEKHKVYACEVTHQGLSSPVTKSFNRGEC

SEQ ID NO: 7 - protein, 120 aa, Artificial Sequence [sequence omitted]

SEQ ID NO: 8 - protein, 451 aa, Artificial Sequence
  Synthetic polypeptide
EVQLVESGGGLVQPGGSLRLSCAASGFNIKDTYIHWVRQAPGKGLEWVARIYPTNGYTRYADSVKGRFTISADTSKNTAYLQMNSLRAEDTAVYYCSRWGGDGFYAMDYWGQGTLVTVSSASTKGPSVFPLAPSSKSTSGGTAALGCLVKDYFPEPVTVSWNSGALTSGVHTFPAVLQSSGLYSLSSVVTVPSSSLGTQTYICNVNHKPSNTKVDKKVEPPKSCDKTHTCPPCPAPELLGGPSVFLFPPKPKDTLMISRTPEVTCVVVDVSHEDPEVKFNWYVDGVEVHNAKTKPREEQYNSTYRVVSVLTVLHQDWLNGKEYKCKVSNKALPAPIEKTISKAKGQPREPQVYTLPPSRDELTKNQVSLTCLVKGFYPSDIAVEWESNGQPENNYKTTPPVLDSDGSFFLYSKLTVDKSRWQQGNVFSCSVMHEALHNHYTQKSLSLSPGK

SEQ ID NO: 9 - protein, 214 aa, Artificial Sequence
  Synthetic polypeptide
DIQMTQSPSSLSASVGDRVTITCRASQDVSTAVAWYQQKPGKAPKLLIYSASFLYYGVPSRFSGSRSGTDFTLTISSLQPEDFATYYCQQHYTTPPTFGQGTKVEIKRTVAAPSVFIFPPSDEQLKSGTASVVCLLNNFYPREAKVEWKVDNALQSGNSQESVTEEDSKDSTYSLSSTLTLSKADYEKHKVYACEVTHQGLSSPVTKSFNRGEC

SEQ ID NO: 10 - protein, 708 aa, Artificial Sequence
  Synthetic polypeptide
MNFGLSLIFLVLILKGVQCEVQLVESGGGLVQPGGSLRLSCAASGFTFADYTMDWVRQAPGKGLEWVADVNPNSGGSIYNQRFKGRFTLSVDRSKNTLYLQMNSLRAEDTAVYYCARNLGPSFYFDYWGQGTLVTVSSASTKGPSVFPLAPSSKSTSGGTAALGCLVKDYFPEPVTVSWNSGALTSGVHTFPAVLQSSGLYSLSSVVTVPSSSLGTQTYICNVNHKPSNTKVDKKVEPKSCDKGGGSGGGSGGGSGGGEVQLVESGGGLVQPGGSLRLSCAASGFNIKDTYIHWVRQAPGKGLEWVARIYPTTGYTRYADSVKGRFTISADTSKNTAYLQMNSLRAEDTAVYYCSRWGGSGFYAMDYWGQGTLVTVSSASTKGPSVFPLAPSSKSTSGGTAALGCLVKDYFPEPVTVSWNSGALTSGVHTFPAVLQSSGLYSLSSVVTVPSSSLGTQTYICNVNHKPSNTKVDKKVEPKSCDKTHTCPPCPAPELLGGPSVFLFPPKPKDTLMISRTPEVTCVVVDVSHEDPEVKFNWYVDGVEVHNAKTKPREEQYNSTYRVVSVLTVLHQDWLNGKEYKCKVSNKALPAPIEKTISKAKGQPREPQVYTLPPSREEMTKNQVSLTCLVKGFYPSDIAVEWESNGQPENNYKTTPPVLDSDGSFFLYSKLTVDKSRWQQGNVFSCSVLHEALHNHYTQKSLSLSPGK

SEQ ID NO: 11 - protein, 708 aa, Artificial Sequence
  Synthetic polypeptide
MNFGLSLIFLVLILKGVQCEVQLVESGGGLVQPGGSLRLSCAASGFTFADYTMDWVRQAPGKGLEWVADVNPNSGASIYNQRFKGRFTLSVDRSKNTLYLQMNSLRAEDTAVYYCARNLGPSFYFDYWGQGTLVTVSSASTKGPSVFPLAPSSKSTSGGTAALGCLVKDYFPEPVTVSWNSGALTSGVHTFPAVLQSSGLYSLSSVVTVPSSSLGTQTYICNVNHKPSNTKVDKKVEPKSCDKGGGSGGGSGGGSGGGEVQLVESGGGLVQPGGSLRLSCAASGFNIKDTYIHWVRQAPGKGLEWVARIYPTTGYTRYADSVKGRFTISADTSKNTAYLQMNSLRAEDTAVYYCSRWGGSGFYAMDYWGQGTLVTVSSASTKGPSVFPLAPSSKSTSGGTAALGCLVKDYFPEPVTVSWNSGALTSGVHTFPAVLQSSGLYSLSSVVTVPSSSLGTQTYICNVNHKPSNTKVDKKVEPKSCDKTHTCPPCPAPELLGGPSVFLFPPKPKDTLMISRTPEVTCVVVDVSHEDPEVKFNWYVDGVEVHNAKTKPREEQYNSTYRVVSVLTVLHQDWLNGKEYKCKVSNKALPAPIEKTISKAKGQPREPQVYTLPPSREEMTKNQVSLTCLVKGFYPSDIAVEWESNGQPENNYKTTPPVLDSDGSFFLYSKLTVDKSRWQQGNVFSCSVLHEALHNHYTQKSLSLSPGK

SEQ ID NO: 12 - protein, 705 aa, Artificial Sequence
  Synthetic polypeptide
MNFGLSLIFLVLILKGVQCEVQLVESGGGLVQPGGSLRLSCAASGFTFADYTMDWVRQAPGKGLEWVADVNPNSGGSIYNQRFKGRFTLSVDRSKNTLYLQMNSLRAEDTAVYYCARNLGPSFYFDYWGQGTLVTVSSASTKGPSVFPLAPSSKSTSGGTAALGCLVKDYFPEPVTVSWNSGALTSGVHTFPAVLQSSGLYSLSSVVTVPSSSLGTQTYICNVNHKPSNTKVDKKVEPKSCDKTHTCPPCPAPELLGGPSVFLFPPKPKDTLMISRTPEVTCVVVDVSHEDPEVKFNWYVDGVEVHNAKTKPREEQYNSTYRVVSVLTVLHQDWLNGKEYKCKVSNKALPAPIEKTISKAKGQPREPQVYTLPPSREEMTKNQVSLTCLVKGFYPSDIAVEWESNGQPENNYKTTPPVLDSDGSFFLYSKLTVDKSRWQQGNVFSCSVLHEALHNHYTQKSLSLSPGGGGSGGGSGGGSGGGEVQLVESGGGLVQPGGSLRLSCAASGFNIKDTYIHWVRQAPGKGLEWVARIYPTTGYTRYADSVKGRFTISADTSKNTAYLQMNSLRAEDTAVYYCSRWGGSGFYAMDYWGQGTLVTVSSASTKGPSVFPLAPSSKSTSGGTAALGCLVKDYFPEPVTVSWNSGALTSGVHTFPAVLQSSGLYSLSSVVTVPSSSLGTQTYICNVNHKPSNTKVDKKVEPKSC

SEQ ID NO: 13 - protein, 468 aa, Artificial Sequence
  Synthetic polypeptide
MNFGLSLIFLVLILKGVQCEVQLVESGGGLVQPGGSLRLSCAASGFTFADYTMDWVRQAPGKGLEWVADVNPNSGGSIYNQRFKGRFTLSVDRSKNTLYLQMNSLRAEDTAVYYCARNLGPSFYFDYWGQGTLVTVSSASTKGPSVFPLAPSSKSTSGGTAALGCLVKDYFPEPVTVSWNSGALTSGVHTFPAVLQSSGLYSLSSVVTVPSSSLGTQTYICNVNHKPSNTKVDKKVEPKSCDKTHTCPPCPAPELLGGPSVFLFPPKPKDTLMISRTPEVTCVVVDVSHEDPEVKFNWYVDGVEVHNAKTKPREEQYNSTYRVVSVLTVLHQDWLNGKEYKCKVSNKALPAPIEKTISKAKGQPREPQVYTLPPSREEMTKNQVSLWCLVKGFYPSDIAVEWESNGQPENNYKTTPPVLDSDGSFFLYSKLTVDKSRWQQGNVFSCSVLHEALHNHYTQKSLSLSPGK

SEQ ID NO: 14 - protein, 469 aa, Artificial Sequence
  Synthetic polypeptide
MNFGLSLIFLVLILKGVQCEVQLVESGGGLVQPGGSLRLSCAASGFNIKDTYIHWVRQAPGKGLEWVARIYPTTGYTRYADSVKGRFTISADTSKNTAYLQMNSLRAEDTAVYYCSRWGGSGFYAMDYWGQGTLVTVSSASTKGPSVFPLAPSSKSTSGGTAALGCLVKDYFPEPVTVSWNSGALTSGVHTFPAVLQSSGLYSLSSVVTVPSSSLGTQTYICNVNHKPSNTKVDKKVEPKSCDKTHTCPPCPAPELLGGPSVFLFPPKPKDTLMISRTPEVTCVVVDVSHEDPEVKFNWYVDGVEVHNAKTKPREEQYNSTYRVVSVLTVLHQDWLNGKEYKCKVSNKALPAPIEKTISKAKGQPREPQVYTLPPSREEMTKNQVSLSCAVKGFYPSDIAVEWESNGQPENNYKTTPPVLDSDGSFFLVSKLTVDKSRWQQGNVFSCSVLHEALHNHYTQKSLSLSPGK

SEQ ID NO: 15 - protein, 15 aa, Artificial Sequence
  Synthetic polypeptide
GGGSGGGSGGGSGGG

SEQ ID NO: 16 - protein, 19 aa, Artificial Sequence
  Synthetic polypeptide
MNFGLSLIFLVLILKGVQC